European Patent Application EP 4 487 866 A1, published January 8, 2025. Title: TGF-β INHIBITION AND ENGINEERED T-CELLS FOR THE TREATMENT OF COVID-19 SEQUELAE AND VIRUS-INDUCED HYPERINFLAMMATION. Applicant: Deutsches Rheuma-Forschungszentrum Berlin. Application EP. The sequence listing filed with the application follows.

SEQUENCE LISTING (3 sequences)

SEQ ID NO: 1 - DNA, 25 bp, synthetic construct
  source 1..25: mol_type = other DNA
ctcaacctggagacaattctactgt

SEQ ID NO: 2 - DNA, 23 bp, synthetic construct
  source 1..23: mol_type = other DNA
tgctagctgttgtccttggttag

SEQ ID NO: 3 - DNA, 16 bp, synthetic construct
  source 1..16: mol_type = other DNA
ctgctgctgctgtttg